European Patent Application EP 4 681 720 A1, published January 21, 2026. Title: Pharmaceuticals for the prevention and/or treatment of diseases or conditions related to reduced blood flow in the brain. Applicant: OSAKA UNIVERSITY. The sequence listing filed with the application follows.

SEQUENCE LISTING (6 sequences)

SEQ ID NO: 1 - DNA, 20 bp, synthetic construct
  source 1..20: mol_type = other DNA
gccagcacataggagagatg

SEQ ID NO: 2 - DNA, 20 bp, synthetic construct
  source 1..20: mol_type = other DNA
aaatgctttctccgctctga

SEQ ID NO: 3 - DNA, 20 bp, synthetic construct
  source 1..20: mol_type = other DNA
gccggcagatgggaatggtt

SEQ ID NO: 4 - DNA, 20 bp, synthetic construct
  source 1..20: mol_type = other DNA
gtctttctcgctgggaccca

SEQ ID NO: 5 - DNA, 18 bp, synthetic construct
  source 1..18: mol_type = other DNA
gcggacccatgggactct

SEQ ID NO: 6 - DNA, 19 bp, synthetic construct
  source 1..19: mol_type = other DNA
ctgctgctgtagtgaccga